European Patent Specification EP 3 365 010 B1, published January 3, 2024. Title: Cytotoxic immunostimulating particles and uses thereof. Applicant: BioNTech AG. The sequence listing filed with the application follows.

SEQUENCE LISTING (1 sequence)

SEQ ID NO: 1 - RNA, 21 nt, Artificial Sequence
  mtiRNA
  misc_feature (3)..(3): 5-fluorouridine
  misc_feature (5)..(5): 5-fluorouridine
  misc_feature (6)..(6): 5-fluorouridine
  misc_feature (8)..(8): 5-fluorouridine
  misc_feature (9)..(9): 5-fluorouridine
  misc_feature (11)..(11): 5-fluorouridine
  misc_feature (12)..(12): 5-fluorouridine
  misc_feature (14)..(14): 5-fluorouridine
  misc_feature (16)..(16): 5-fluorouridine
  misc_feature (19)..(19): 5-fluorouridine
  misc_feature (20)..(20): 5-fluorouridine
aguguuauucuuguaugguug